European Patent Application EP 4 438 739 A1, published October 2, 2024. Title: 基于重组酶聚合酶扩增技术的逆转录扩增系统和方法. Applicant: 广州达安基因股份有限公司. Application CN. The sequence listing filed with the application follows.

SEQUENCE LISTING (4 sequences)

SEQ ID NO: 1 - DNA, 305 bp, Homo sapiens
  source 1..305: mol_type = genomic DNA
cagtgtatctggaaagcctacaggacaccaaaataaccttaatcatcaattggttacaggaggctttaagttcagcatctttggctcacatgaaggccaaattccgagagactctagaagatacacgagaccgaatgtatcaaatggacattcagcaggaacttcaacgatacctgtctctggtaggccaggtttatagcacacttgtcacctacatttctgattggtggactcttgctgctaagaaccttactgactttgcagagcaatattctatccaagattgggctaaacgtatgaaagca

SEQ ID NO: 2 - DNA, 33 bp, synthetic construct
  source 1..33: mol_type = other DNA
cagtgtatctggaaagcctacaggacaccaaaa

SEQ ID NO: 3 - DNA, 32 bp, synthetic construct
  source 1..32: mol_type = other DNA
tgctttcatacgtttagcccaatcttggatag

SEQ ID NO: 4 - DNA, 51 bp, synthetic construct
  source 1..51: mol_type = other DNA
attcagcaggaacttcaacgatacctgtctctgtaggccaggtttatagca